European Patent Specification EP 3 891 288 B1, published October 9, 2024. Title: MATRIX ATTACHMENT REGIONS AND USES IN PROMOTING GENE EXPRESSION. Applicant: Celltheon Corporation. The sequence listing filed with the application follows.

SEQUENCE LISTING (36 sequences)

SEQ ID NO: 1 - DNA, 186 bp, Artificial Sequence
  Synthetic
aaataattaattagcaaataatttatatatttatatatttatatatatatatatatatatatatatatatatatatatatatatatatatatatatatatatatatatatatatatatatatatatatatatatatatatatatatatataaatatataaatatatatatatatatatatattggt

SEQ ID NO: 2 - DNA, 185 bp, Artificial Sequence
  Synthetic
aaatatttcaaaaattaagcaaagaaactttcacagtatgactaataatattttttcttctggagaaagtcttatttgtcttatttcggctagaataaaaacagtttttaattttttaaacaccattttacggacaaaattattagcccctttaagctatatttattttcaatagtctacagaac

SEQ ID NO: 3 - DNA, 98 bp, Artificial Sequence
  Synthetic
gggagaagcagtccaatgtggctgtatatatatattattatttttttttttttaaatacaaacaattaagctgtcgaactgttgtataaacacaatat

SEQ ID NO: 4 - DNA, 1879 bp, Artificial Sequence
  Synthetic
atgcaaaggactctttctgtaaaatatctgctgtaaaaatctaaaggatttgagggttgcactcccaaaggctcctgagagcttgtgtaaaataagccttcctaactgctgctttctcactttagtcaattttggccttttttatattcatatacagtaaatgttgctctaatcaatgtggatgatcattatcagtatatgactcgaaaaatattttaaacttctctttgcttctagaccaggatttgaaggaatattctatttttaatgacactgctttgcaatatttatgattcttaaagtcaaacagagtgaaacagaagtaaacatgtcatgatgtacactcacatgaaacaatctctgaaatgaagaatgaatgaagaaagttgtgttgctaacaaaatggaggaagactcacgaatagacaaaagcagggcagaaacgagacacgcacccgtgtacatatatacagttgaagtcagacttattagcccccctttgatttttttttctttttttaaatatttcaaaaattaagcaaagaaactttcacagtatgactaataatattttttcttctggagaaagtcttatttgtcttatttcggctagaataaaaacagtttttaattttttaaacaccattttacggacaaaattattagcccctttaagctatatttattttcaatagtctacagaacaaataattaattagcaaataatttatatatttatatatttatatatatatatatatatatatatatatatatatatatatatatatatatatatatatatatatatatatatatatatatatatatatatatatatatatatatatatataaatatataaatatatatatatatatatatattggtgggagaagcagtccaatgtggctgtatatatatattattatttttttttttttaaatacaaacaattaagctgtcgaactgttgtataaacacaatatcactcgagttgcagtccgatgtgactatatattggcactggtgggagatttgcattcattgtgacaatatacagccacattgcattgctacgagtgtgatattatgtttatacaccagttcaacagcataatcgtgtgtaataaaaagataatcaaacacggaagaggaactactttcttccgccattcattcacatctgcagcttacgtcagaacagcagaagctgttgctcattcatatatataatatatataaatttgtatacttacagacgacacagtggctcagtggttagcactgtctcctcacagcaagaaggtcactgtttcaagtccaggctgggtccgccggcatttgtgtgtggagtttgcttgtttttcccgtgttaatgtgtatggatgtttcccagtactgggttgcagctggaagggcatccgctgtgtaaaacttatgctggataagttggcagttcattccgctgtgtcaacccctgatgaataaagggattaagccaaatgaaaatgaatgaatgatttaatactcttgtttaagtcttagtgccgattatatatagatatgtggtgttagatcaaaccagtgttcattttgacagcaaaatttgatttagttttagtcattttttagtcttccatattcgttatagcatcagtctatatacagtcaactaaattaaacatgattttagtcaacttcatgcattttcacatggacaaggtcattaaaattctacaggatcaggttgtaccaactctatctcatggaaatttgtaactttttgattgtggctaattcgtatgaatttgtatgatctcatttgtacaatttagtattatttgctcatcccccagtgatggttggatttagggttg

SEQ ID NO: 5 - DNA, 225 bp, Artificial Sequence
  Synthetic
tatccaaatatatatatatatatatatatatatatactatatatatatatatatatatatatatatatatatatatatatatatatatatatatatatatatatatatatatatatatatatatatatatatatatatatatatatatatatatatatatatatatatatatatatatatatatatatatatatatatatttttttttttttttttaagaaaaca

SEQ ID NO: 6 - DNA, 106 bp, Artificial Sequence
  Synthetic
caaatttgctatacaaaaacctaaatgtaataaagttacatccataaaagtgactttttattacttttgaaacacaacagatttatgccctgtctatatccagttc

SEQ ID NO: 7 - DNA, 109 bp, Artificial Sequence
  Synthetic
gttataataattttataatctctcacaatattgctgttttactgatttttgaataaatgcagccttggtgagcataagagactttttctaaaaactttgaaaagtctta

SEQ ID NO: 8 - DNA, 2679 bp, Artificial Sequence
  Synthetic
tgttacattaggctgaaaacacactgtgtatgtgcatattttcccttaaatacataaagaagtaatgggtggcgtacctgtattggttatagactccagggcagtataacatggctgtgaatagactctgttgtggacatacactccataacaccaaactgatcccgtagaacgatgtcaccaggaaaagaaggagcgtcaaaatgaactgcctgtgattggcttgacctacacagctgtttatcctgtcatggaaagtcacatacatacaagacacaaataataagcaacacatttacagatattttcattcaaacaatttagaacaattatactattttctctcttgtcaatgtagctttaatgagaattatgtggctcatggcatgttcatatttatatttgtgcctgtgtgtgtgttgaagtagcatggagacagattggcctggtgagagctccctttactgtgctgaaaactgtgttcctgttgcctttgcacatgtctcaccagcctgcctgctccagtgacgtcttttgggaatcagcttgaacatatgtgtgtgtctgatggggtagggaacacatgcatacaagtgtgaagagatcagaaaatgaatcaaatcattggcatgaccactaatttaaacaattcattttggaattgttcagctacttctgtagtaaggatttgcaataagccagatatcttagaaggaaaggcacaaatatcaacattaaaattaatatttgaaataacagaaaatatattcggttgactgattatccaacaaacacaagtgtaaagtgatatttttaatgaacatctaaaattacaatgcaacggtaagtctgtgaagctgagatgattaaaatgtgatctttatgaatgaaagcagatggccacaatgctctctctccttttattgtttataaatcataaatcatcaattcatatagtaacttttttagattttgaatatttatttatgtaaagttttaaatattattgaatagtaaataatttaatatgataatcatttataaaagtgtatatttgtaaatacaattatttttaaaatatataaatgatgaaaaaaatttaaatataagaataaacacttttataaataatacaaggcaaatttgctatacaaaaacctaaatgtaataaagttacatccataaaagtgactttttattacttttgaaacacaacagatttatgccctgtctatatccagttctatccaaatatatatatatatatatatatatatatactatatatatatatatatatatatatatatatatatatatatatatatatatatatatatatatatatatatatatatatatatatatatatatatatatatatatatatatatatatatatatatatatatatatatatatatatatatatatatatatatatttttttttttttttttaagaaaacagttataataattttataatctctcacaatattgctgttttactgatttttgaataaatgcagccttggtgagcataagagactttttctaaaaactttgaaaagtcttaccgacaacatattattgaatggcagtgtaaatatagatcgttttgtcatttagagaatatttaattaatgtttaatacacttcacactaggaatgaagtgctcgtactcaatttttaaagaagaaggaatgagaaacccaccaaacacagtggtggtccattcgaaggacacatgccccacagatcctgcagtgccctgcccttggtgggcgcacctgtcggcacacagggcataacttcttctttccttcgttttccccatttgactgactgattcctttgcagggggcggagtctccaggtatgtttgtgctctgattggttgtacagatactgttaattccctgagctaatgactgggatttgacaaagcctggtccttgtttggtgcgcacaagggagataagggtcaacatcatgcctgtcgtcacagtaaccagctgcagattactgacgtctcctctgggaacgatctcagtaaggaaaagatagtacatgtaggcaagggagaaaagtgccaagctaaggaaaaacaatgtgcgtcttttccttctgtgagtcacatagtaataccaaagcaccagtcctggtagggcagttaggacaacaactcccaacatacagttaattgctgctactcgcaacagaccaggaattaataccatgggaggtaagacagagatttccaatcgaaggggtcctacggcacaacatggcaaacccaaacgatcagccatacaagagacgaaacgagagaagatgtctggcttgtcttgctctcctctgactaacctattgagaaagagtgacaaattcaccattcatcatttacacactattatgttatcagttttatgtatggaaatgacaaggtgcaaacggacaaaattatttaattcaactacactttttaaagtgtaaaaatgtaaagtgtcaaaagtttatatcaataaatgtaatgtaaaaccatctctgcatgccatgatcttaactggttgacctctgacctttcacaggcatcatctagttcttcacagtcacagcagcagtactctctttgctggtcgatgtctccacagcagcacagagggtcatctggtt

SEQ ID NO: 9 - DNA, 350 bp, Artificial Sequence
  Synthetic
atatatatatgttagtgatatatatataaaatatatatcactcttattatatattatatatattatataatatataatatattatattatataatatattatatattatataatatatataatatattatatattatataatataatatattatatattatataataatataatatattatatattatataataatatataatatattatataataatatataataatatataatatattattatataatatataataatatataataatataataatgtgattatattatatataatatgtaatataataatgtatatatattatatatgcattatatataatgatttt

SEQ ID NO: 10 - DNA, 186 bp, Artificial Sequence
  Synthetic
aattgcataagccaatcccttgcaataaataaaatagatcgagatgtagatagacagagatccagatcctactggttccattttcctggcagaaccatgatggatatgatatatgtcccataaagagcctcccagtggtgtctttttgttttgtaaagatggttttaatccacagatttaagagtg

SEQ ID NO: 11 - DNA, 153 bp, Artificial Sequence
  Synthetic
ctatcaaatgtatatttaaatctacctacttgtgttatatatttatatatgtgtgtgtgatatgtataattttaaaatatatctgtatagctacttaatttgtatttccagcccaattcagtctagtgacagaaaatataactcatcaagtct

SEQ ID NO: 12 - DNA, 4061 bp, Artificial Sequence
  Synthetic
tacccagtaattcttaaactacttactccagcacttggcccatggcaaatttcctggtagccatatgtacatatacacatgcttttaaatacataaacgtatgtacatatacttttaatttactactaagattttatacattttccagtagtttgtatgatgaacatgtatatacctccctttaaagttaaacaataaaaaaatcttaatttttctaccttaaaatctcctctcatcacgtcatccaatgatagccgctgttaacatcatgttcctatttacttctgcttgtttctctgaagatgtacgtgagtgggtaaacacgatgtaatttgacattgcggtttttaatagcatatcacaaatattttcctgttataatttcattcacaaacatggttctgatagttacataatattacaccatatgatcatttcctagtttacttagctatttcctatggttggatattcttggcttgtttccaatatttttctattctaattcatctccaacaaaagtcatcatctgtgaatctttctctgcatctctaagtatttccttagaataaactcctagagtgaatctgttagcacatttgtttctctcttttaattaacaactggaaaatgattattgcagacacattctcttcaagtgaatatttcttctcggctgaactttgctttactgagtatttttccctcccttggctgcattttcattcttcttttgctgttttgcgtttcactcccacctacaaaatatccaagttccctctcccaaaataaaacccctcttggttcatggcagagtcaactttgttcagctgtctttaccctgcaggtccaaaggtctattgcccagagtatttgctgaggggataagaggtgccaggtcctcatcagagtaatctttgcatcttccattttagatgatgaggctgaggctaaataactttttgtgacttgaacaaaatcacgcccgtcattttggagcagagattggacccagaccatctgactgcagtgcacttggttactacacaacagccctggaagctgcaacctgaggacctccagcctcacatgaatcatcttcatccaccaaccttctcccatctgggttcccacactcctcccatcacccagcatggggggcctcatggtggtggttgacccttcctctatctccacctgcatatggggcacattctccccaaacctcactccagtccaatctcacctcaaccccactgtctcgctcatagggttgaggaaagacagaataaaccctggctgggaaaagtcactttagtcaatgtacggtcagttttacgtgtcagcttggccaggctagagtccccagtcatccaaacgcccagttgactgtaagcaaagactatcctagataatttggtcggcctgagacattcagttaaaagaccataagagcagaactgaaaacagaaaattctgcctgtggactgcagcgccagctcctgcctgagagtttccagcctgaccttcctaaacttgcctactaatcccccacaattgcataagccaatcccttgcaataaataaaatagatcgagatgtagatagacagagatccagatcctactggttccattttcctggcagaaccatgatggatatgatatatgtcccataaagagcctcccagtggtgtctttttgttttgtaaagatggttttaatccacagatttaagagtgatatatatatgttagtgatatatatataaaatatatatcactcttattatatattatatatattatataatatataatatattatattatataatatattatatattatataatatatataatatattatatattatataatataatatattatatattatataataatataatatattatatattatataataatatataatatattatataataatatataataatatataatatattattatataatatataataatatataataatataataatgtgattatattatatataatatgtaatataataatgtatatatattatatatgcattatatataatgattttctatcaaatgtatatttaaatctacctacttgtgttatatatttatatatgtgtgtgtgatatgtataattttaaaatatatctgtatagctacttaatttgtatttccagcccaattcagtctagtgacagaaaatataactcatcaagtctgggtaatctcaaataattcggctaaattcctcaattcatcaatttctccctcctccagcctccgcataattgattctaactttcagggagttgaagcagcactgccctggggggctctcttccagctctcagcccctccctgcacagctctggtgcccacggggatgcgcccacggggatgcaaggccctgtatgaccatcagacctcctgtcctcacttgagatgtttatttctagtccccagtcctgccccaaccacaggatgtaacccagaccctggtctctattccaagattcatccttgtcaagcggttctcagcagcatgcctctgccacgcccagtcacagaggacgatattggctcccctctttatggggggaggataaaaaggatcatatcccagacccctgggcttaaggcttccatgttcccatctctactctttaatgccaggatgacatagggtactttctgcaggcatagacaaccaggcaggaagaggggcccatgttccttgtaatctcagatcacaagtaccctctggggatctatcaccccaagcttggtgcatggacaaggggtaccttattctcttcctttcttctaagactatgcactgcctctcccccaggcaaatggaatcttgtcaattccaagtgagtttggaaaaactcattcttttttacttattgtttagatcggaacctaaaatcgaaagttccaggaagctcaagttcttataactaaaaaggcttttctctctcaagagcattggctctgtcttttccatgttctactttgaaacacaaaagctgagctcgacattgatttaattgctttttatttgaatgattgctataagtgacaccttttggggcagtatgtcctagctggttgaattagagttgggaaacacattgcaagaaagggtagaaagaggcatactttattgaatcttttggagtaacttttgtgcctgttaccacaagcttatttttgataagatgcttcctaactttcctcgctcacccctacctcatctcagggccaagcacgaaagttgttttatacatgctaggtttggctgatttcaatgtgacttccccagggcagaagagacagtggttgaaggatgaagaatcaacctacccgggggaatcaaagattgatcccagggaatggagcagatataattaaataagttttttctttccccagtgtatctaatattcatttttgtatttacttggagcaaatgaatttaaatgaatttttagttagagttaaatcaactcattaaaacacattgaaggaattagaaatgtaaaatcatttcctgctgcaattcattcatctctaagtctataactgacttgaatctaggtaaaggtcattgcttaaaggggacagtggcccttattcttgcaacctacaaacttttacagtttgcatggagttttcacatccatgaactcaagcaagactgaataggcctgtatggtgaacaaacaggagtaaatgcctccactattcaggggaggaaagtgagctcaaaaaagtttaatattgttgcctaaggatactcaaccagcaaatggcaatatcgagacaggagcaggtcttcagtccaaacccacagagcagagcttgcccaggaagctgatcattcttgtaccaccttctccatcactggacctacaccctgcccttctttacccagctctgacctctcagatgctgaacctggggtgcccttgtcattgaacttcgagttgcattattttcccattgttttacctacaattaacttgccgtc

SEQ ID NO: 13 - DNA, 1700 bp, Artificial Sequence
  Synthetic
agactctgtctcaaatatatatatatttatatatatatattttatatttaatatatataatatatattatatataaatttattatatataatatatattatatataaatttattatatataatatatattatatatattatatgttatatatatttattacatataatatataatatatatttattatatataatatatatttattatatattatatattatatattttatattttatatatattatataattttatattttatatatattatataattaatatttaatatatattatatatatatatataatatatatttattatatataatatatatttattatatattatatattatatatttatattttatatatattatatatttatattttatatatattatatatttatattttatatatattatatataatatatatattatatattttatatataatatatatttattatacatattttatattatatataatatatatttattatatatttttatatatattatatataatatatatatatttatatatatatattttatatttaatatatataatatatattatatataaatttattatatataatatatattatatataaatttattatatataatatatattatatatattatatgttatatatatttattacatataatatataatatatatttattatatataatatatatttattatatattatatattatatatttatattttatatatattatatatttatattttatatatattatatatttatattttatatatattatatataatatatatattatatcttttatatataatatatatttattatacatattttatattatatataatatatatattatatatatatatatatatatatttatatatatatatatttatatattttatatatatataatatatattaattatatataatatatatattatatatatattatatataatacgtaatatatatttattatatatattttgtatatattatatattatatatttattatatatattttatatatattatgtatattttatatacaatacataatatatattttatatacaatatataatatatattttatatacaatatataatatatattttatataatatatttttatataatatatattttatattatatataatatatattttatatattatatataatatatattttatattatatataatatatattttatactatatataatatatattttatacattatataatatatattttatactatatataatatatattttatacattatataatatatattttatatattatataatatatattttatgttatataatatatattttatgtattatataacatatattttatgtattatataacgtatattttatatattatgtaacgtatattttatatattatgtaacgtatattttatatattatgtaacgtatattttatatattatgtaatatatattttatatattatatattttgtatattatatattttgtatatgatatattatatattttatatattatatattatatattttgtatattatatattatatattttatatataatatatcatatatattttatatatatataaagcatcagtaaacaa

SEQ ID NO: 14 - DNA, 177 bp, Artificial Sequence
  Synthetic
taacatggtgaaatatcatctctactaaaaatacaaaaaattagccaggcgtggtggcgggcgcctgtggtcccagctacttgggaggctgagggaggagaatggcgtgaacccaggaggcatagcttgcagtgagccgagattgcaccactgcactccagcctgggcaacagagca

SEQ ID NO: 15 - DNA, 249 bp, Artificial Sequence
  Synthetic
ctctagagccaggcaccgtgactcactcctgtgatcccagcttttcgaaaggctgaggcaggaggatcgcttgaggccaggagttcaagaccagccttggcaacatagtgagactctcccgtctctaaaacaacaacaacaaaaggttaattaaaaattaaaagaaaagaaaactccacagccaccttctccaggaaaataagtcccaaagccacttgccactgatgcagaggtgcgcagagcccgagg

SEQ ID NO: 16 - DNA, 5274 bp, Artificial Sequence
  Synthetic
gacagatgggattattcatttttataaaatatttaacccaacaaatccaaaatatcatttcagcatgtaaataatacagatggtccccaatttaaccatggttccattaaaggattttttttgactttaataatggatttatcagaatataacctcatcataagttgaggaacatctgtataaaaatatattaatgagataccctacattcattatcctttgtataccaagtcttaccatgtggattttgcacttcccacacatctcaatatggaccagccatatcacgtgccccctgccagatgcatctagtggctttcacatcggacagctccacactagaatgacagtaaggcacagaaccagacagtccccccgcttccagctcctgatcaaccacttgtagccatgggagctttggagactgccttaatagttatgaatctaagctaggtgtcatggctcacacctgtaatcccaactctttgggacgccaagatggatggatagcttgaggctttttttttttttttttttttttttagacaagagtctcgctctgttgccaggctggagtgcagtggcacgatcttggctcactgcaacctccgcctcccaggttcaagggattctcctgcctcagcctccccctgagtagctgagactacaggtgcgcaccaccacgcccagctaatttttgtatttttagtagagacagagtttcaccatgttggccagaatggtctcgatcacttgacctcatgatccacccacctcagcctcacaaagtgctgggattacaggcgtgagccaccgcgcccggccagcttgacgcttgagtccaggaattcaagaccagcctgggcaacatggtcgaaaccctgtctctactgaaaaaaaaaaaaaaaaattatccgggcatggtgacacacgcctacagtcccagctaccccagaggctgaggtgggaggatcattgaacccctaaaagtcaaggctgaagtgatccaagattgcatcactgaactccagtctgggtgatgggagtgagaccctgtctcaaaaaaaaaaaaaaatagaaaagctctgaatctatgggttctagccctgggaaattctggataacatggagttaacagttcacctgcctcaggtgagataatgtaaaactagaaaggtccataccattgtgatgtctaattgaatctatttatcaaaacagtacccaaatgcagtatgttcagaaaccttatactgttaggtaataataaccataaacaagataaaaaatatgggctgggtgtggtggctcccactgttatcctagcattttgggaggcgaaggcaggaggatcacttgaggctgggagtttgagaacaacctgggcaacatagcaagaccccatctctataaaaaaacatataaatataatataaagatatatatattttatatatatacatatatttgtacctgttaacgtggggtgaggggtgcagggagggtggaaaggagaaagtcataatattaagcatcagtaggccgggcgcagtggctcatgcctgtaatcccagcactttgggaggctgaggcgggcagatcacaaggtcaggagattgagatcatcctggctaacatggtgaaatatcatctctactaaaaatacaaaaaattagccaggcgtggtggcgggcgcctgtggtcccagctacttgggaggctgagggaggagaatggcgtgaacccaggaggcatagcttgcagtgagccgagattgcaccactgcactccagcctgggcaacagagcaagactctgtctcaaatatatatatatttatatatatatattttatatttaatatatataatatatattatatataaatttattatatataatatatattatatataaatttattatatataatatatattatatatattatatgttatatatatttattacatataatatataatatatatttattatatataatatatatttattatatattatatattatatattttatattttatatatattatataattttatattttatatatattatataattaatatttaatatatattatatatatatatataatatatatttattatatataatatatatttattatatattatatattatatatttatattttatatatattatatatttatattttatatatattatatatttatattttatatatattatatataatatatatattatatattttatatataatatatatttattatacatattttatattatatataatatatatttattatatatttttatatatattatatataatatatatatatttatatatatatattttatatttaatatatataatatatattatatataaatttattatatataatatatattatatataaatttattatatataatatatattatatatattatatgttatatatatttattacatataatatataatatatatttattatatataatatatatttattatatattatatattatatatttatattttatatatattatatatttatattttatatatattatatatttatattttatatatattatatataatatatatattatatcttttatatataatatatatttattatacatattttatattatatataatatatatattatatatatatatatatatatatttatatatatatatatttatatattttatatatatataatatatattaattatatataatatatatattatatatatattatatataatacgtaatatatatttattatatatattttgtatatattatatattatatatttattatatatattttatatatattatgtatattttatatacaatacataatatatattttatatacaatatataatatatattttatatacaatatataatatatattttatataatatatttttatataatatatattttatattatatataatatatattttatatattatatataatatatattttatattatatataatatatattttatactatatataatatatattttatacattatataatatatattttatactatatataatatatattttatacattatataatatatattttatatattatataatatatattttatgttatataatatatattttatgtattatataacatatattttatgtattatataacgtatattttatatattatgtaacgtatattttatatattatgtaacgtatattttatatattatgtaacgtatattttatatattatgtaatatatattttatatattatatattttgtatattatatattttgtatatgatatattatatattttatatattatatattatatattttgtatattatatattatatattttatatataatatatcatatatattttatatatatataaagcatcagtaaacaactctagagccaggcaccgtgactcactcctgtgatcccagcttttcgaaaggctgaggcaggaggatcgcttgaggccaggagttcaagaccagccttggcaacatagtgagactctcccgtctctaaaacaacaacaacaaaaggttaattaaaaattaaaagaaaagaaaactccacagccaccttctccaggaaaataagtcccaaagccacttgccactgatgcagaggtgcgcagagcccgaggaacacggagtcatagcagctctgcaaattgattttattccaggctaaaagatgctatttctcaaaaaaaggagctgggagcgtctctgttcatgaattcatttttcaggggtggggtgatttcaagagtccaggctgtttcctgaccatgcacactgttccggcctggaagcctcagaccccagccaggctgaccacgagccagacccggagtaagcttcgtcccatgcttcctgtcggtccgggcagcctgagtttcctggtgacccttccctgcacccagccaattcaaaggtctggcaaggcctggtgccagccaagaaaatctgaggcagccaggtttgttatttcaaatctctaaaccttcagacctctgtgcttggcttacatatgtgaaagttaaaacaaggatgtgtgtcgcagtggtgattataattcaagtaagcaaagatccctgcatgaccagccttcgaatgtcagcccatgctgaagttaacacatttaactcatagaacaaaatagttaaaatgaggagtggatgcaaaatggtactgccattctagaaaacagttggcagtttcttataaagttaaacgtacgcttaccacaagacccagcaatcaccctcccagagaaatgaaaatttatgttcatataaaatattgtacacaaataattataacagctttatttgtaatagtcatgtatcaatcaggattctccaaggaaacaggaccaatagaagagagatatatacataataaatcatatatataaatgatatatataagaagttatatatatatacacaaacacatacatatattgtgataacctaccttgttttaacctgagtgactctctcctagcagagagagccagacagactccattttagtttcttcattcacagccccctttatcccccttaagggaataactagtgcaagctgactctaagcacatccagtaatgcacctgctgataagatattgaggcaggctgtaccagcagctcctgggaatgtgctcggtggaaggtatctaaaagcccctgcatttatctcttagtgatagtttaagcccctgcacctggaactgtttatcttttacaactgcttctataaccaattaattttttaactttttgcctgttctgcttctgtaaaactgcttcagttaaactccccctcccctatttagaccatagtataaaagagaatctagccccttcttcggggctgagagaattttgagtgctagctgtctctcagtcgccggctaataaaggactccataatttgtctcaaagtgtggcgtttctctataactcgcttggttacaacactatctctcagggatctccaaagaaatagaacctataggatatatctatctataataaatcattgccaggcatggtggctcacccagtactttgggaggccaagtcaggaggatcacttgagcccaggagtttgaggccacctgagcaacatagtgagaccctgtctctac

SEQ ID NO: 17 - DNA, 965 bp, Artificial Sequence
  Synthetic
ccagctactcgggaggctgaggcaggagaacggcttgaacccaggaggtggaggttgcagtgagctgagatcgcgccactgcactccagcctgggcgacagagcgagactctgtctcaaaaaaaaaatatatatatatatatatatacacatatatatataaaatatatatatatacacacatatatatataaaatatatatatatacacacatatatataaaatatatatatatacacacatatatataaaatatatatatacacacatatatataaaatatatatatacacacatatatataaaatatatatatacacacatatatataaaatatatatatacacacatatatataaaatatatatatacacacatatatataaaatatatatatacacacatatatataaaatatatatatacacacatatatataaaatatatatatacacacatatatataaaatatatatatacacacatatatataaaatatatatatacacacatatataaaatatatatatacacacatatataaaatatatatatacacatatatataaaatatatatatacacatatatataaaatatatatacacacatatatataaaatatatatatacacacatatatataaaatatatatatacacatatatataaaatatatatatacacatatatataaaatatatatatatacacatatatataaaatatatatacacacatatatataaagtatatatatacacacatatatataaaatatatatatacacatatatataaaatatatatatacacatatatataaaatatatatatacacatatatataaaaatatatatatatattttttaaaatattccaattgtctcactttgtggatgagaaaaagaagtagttagaggtcaagtaacttggcctacatcttttctcaagattgtaaactc

SEQ ID NO: 18 - DNA, 256 bp, Artificial Sequence
  Synthetic
ctgtgctcccttaacatcctattttatctgtatatatatatattcttccaaatatccatgggaaaaaaaatctgatcataaaaatattttaggctgggagtggtggctcacgcctgtaatcccagcactttgggaggctgaggtgggcggatcatgaggtcaagagatcgagaccatcctgaccaatatggtgaaaccccatctctactaaagatacaaaactattagctggacgtggtggcacgtgcctgtagtc

SEQ ID NO: 19 - DNA, 240 bp, Artificial Sequence
  Synthetic
ctagtgagcaataaccacatcttcattttctttgtataaaacaagaaagtttagcatgaaaaaggtactcaattacaaatgtgttggattgaattgaagacccttggaaggggattttgtacctgaggatctctttcttttggccatattgttcaatggacaaaatttagccttcgaaggcaggccgatttgaggttaatactacctttaccacttgatagctatgtgaccttggccatg

SEQ ID NO: 20 - DNA, 3612 bp, Artificial Sequence
  Synthetic
gactctagattataccaacctcataaaataagagcatatataaaagcaaatgctcttatcttgcagatccctgaactgaggaggcaagatcagtttggcagttgaagcagctggaatctgcaattcagagaatctaagaaaagacaaccctgaagagagagacccagaaacctagcaggagtttctccaaacattcaaggctgagggataaatgttacatgcacagggtgagcctccagaggcttgtccattagcaactgctacagtttcattatctcagggatcacagattgtgctacctattgcctaccatctgaaaacagttgcttcctatatttcatccagtttaatatttatttaaaccaagaaggttaatctggcaccagctattccgttgtgagtggatgtgaaagtaccaattccattctgttttactattaactatcctttgccttaatatgtatcagtaggtggcttgttgctaggaaatattaaatgaatggcatgtttcataggttgtgtttaaagttgttttttgagttaaatctttctttaataatactttctgatgtcaaaaacacttagaagtcatggtgttgaacatctatatagggttggatctaaaatagcttcttaacctttcctaaccactgtttttgtttgtttgtttttaactaagcatccagtttgggaaattctgaattaggggaatcataaaaggtttcattttagctgggccacataaggaaagtaagatatcaaattgtaaaaatcgttaagaacttctatcccatctgaagtgtgggttaggtgcctcttctctgtgctcccttaacatcctattttatctgtatatatatatattcttccaaatatccatgggaaaaaaaatctgatcataaaaatattttaggctgggagtggtggctcacgcctgtaatcccagcactttgggaggctgaggtgggcggatcatgaggtcaagagatcgagaccatcctgaccaatatggtgaaaccccatctctactaaagatacaaaactattagctggacgtggtggcacgtgcctgtagtcccagctactcgggaggctgaggcaggagaacggcttgaacccaggaggtggaggttgcagtgagctgagatcgcgccactgcactccagcctgggcgacagagcgagactctgtctcaaaaaaaaaatatatatatatatatatatacacatatatatataaaatatatatatatacacacatatatatataaaatatatatatatacacacatatatataaaatatatatatatacacacatatatataaaatatatatatacacacatatatataaaatatatatatacacacatatatataaaatatatatatacacacatatatataaaatatatatatacacacatatatataaaatatatatatacacacatatatataaaatatatatatacacacatatatataaaatatatatatacacacatatatataaaatatatatatacacacatatatataaaatatatatatacacacatatatataaaatatatatatacacacatatataaaatatatatatacacacatatataaaatatatatatacacatatatataaaatatatatatacacatatatataaaatatatatacacacatatatataaaatatatatatacacacatatatataaaatatatatatacacatatatataaaatatatatatacacatatatataaaatatatatatatacacatatatataaaatatatatacacacatatatataaagtatatatatacacacatatatataaaatatatatatacacatatatataaaatatatatatacacatatatataaaatatatatatacacatatatataaaaatatatatatatattttttaaaatattccaattgtctcactttgtggatgagaaaaagaagtagttagaggtcaagtaacttggcctacatcttttctcaagattgtaaactcctagtgagcaataaccacatcttcattttctttgtataaaacaagaaagtttagcatgaaaaaggtactcaattacaaatgtgttggattgaattgaagacccttggaaggggattttgtacctgaggatctctttcttttggccatattgttcaatggacaaaatttagccttcgaaggcaggccgatttgaggttaatactacctttaccacttgatagctatgtgaccttggccatgtggtttcaacagtctgaacctcattttctctgtgtatgtgtggtcctccttacaagtttgtgaaaaatgtgaagtccttagccatgatagcccaatataacaggctaaatgataataggtttatgttcttttcctttatattctcagataagcactgtccaagtttgaggtgttttgaggtctcgcctgatttggattgtttgagtttatgctattctttgaattctttgagctgttctgaagcagtgtatcatgaacaaaaacatccccagttcagtccaaacccctggttacatatcattcttatgccatgttataaccagtttgagagtgttccctctgttattgcatttaagtttcagcctcacacagaaattcagcagccaatttctaagccctaagcataaaatctggggtgggggggggggatggcctgaagagcagcattatgaatagcaccattataattaatgatctctcaggaagatttacaatcacaggtagcagataaaacaaatagtactgcttctgcacttcccctccttttattcgctatgaaattttatgggaaatcagtccagtgaaaaatgtaagctcttaatctttcccagaaatcctacctcatttgatgaatactttgagggaatgaattagagcatttttttcttttatagtctacttcgcatttacgaagtgaggacggtagcttaggctgcctggccaactgatgagaaggtcagaggcatttttagagacctctgttgtctttcattcatgttcattttccacaaggcaagtaatttccaacaaatcagtgtcttcattagtaataagattattaacaacaataatagtcatagtaactattcagtgagagtccattatatatcaggcattctacaaggtactttatatacatctgagtaaacctcacacaattctacagggaggtatttctatccccatttaacaaataaggaaacgaagtccaagtaaattaacttgcccaaggtcacacagatagtacctggcagaacaggaatttaaacctaaatttgtccaactccaaaagcagccttctatttgttataaatgctgcctctcattatcacatattttattattaacaacaacaaacataccaattagcttaagatacaatacaaccagataatcatgatgacaacagtaattgttatactattataataaaatagatgttttgtatgttactataatcttgaatttgaatagaaatttgcatttctgaaagcatgttcctgtcatctaatatgattctgtatctattaaaatagtactacatctagag

SEQ ID NO: 21 - DNA, 599 bp, Artificial Sequence
  Synthetic
atatgtatatatgtatatatgtatatatgtatatatgtatatatgtatatatgtatatatgtatatatgtatatatgtatatatgtatatatgtatatatgtatatatgtatatatgtatatatgtatatatgtatatatgtatatatgtatatatgtatatatgtatatatgtatatatgtatatatgtatatatgtatatatgtatatatgtatatatgtatatatgtatatatgtatatatgtatatatgtatatacgtatatatgcatatacgtatatatgtatatatgtatatatgtatatatgtatatatgtatatatgtatatatgtatatatgtatatatgtatgtatgtatgtatgtatgtatatatgtatatatgtatgtatgtatgtatgtatgtatgtatgtatatatgtatatatatatgtatgtatgtatgtatgtatgtatgtatatgtgtatatgtgtatatgtgtatatgtgtatatgtgtatatatgtatatatgtatatatgtatatatgtatatgtgtatatgtgtatatgtgtatatatgtatatatgtatatatgtatatatgtatatatataacat

SEQ ID NO: 22 - DNA, 205 bp, Artificial Sequence
  Synthetic
gctctttcctttagttaagcttatgaaatagtgtttctctcatgtttcctctatattctctcttttgccttcctgtttcttcctgttgattccatcccattggagtgaaatcttatgatcttttggcatcaacaaagtgatctgcatccaaataattccacatctcattccatgttgactgtggatctatatatatatatatgta

SEQ ID NO: 23 - DNA, 352 bp, Artificial Sequence
  Synthetic
agtattaaattatatatacatatataagtgaaatgtcacaatcttctagaacttgctctgtatgtccacttaacatggtagagtgagctatgtcagcattttctatttcctgtgaatcattctgtgtgttgccaagaagaaatatgatatattctgaggttatgaaatgatattttggtcatcatgtttctcatcctattttcatattacctaaatacttttgcttttaaaattattattattaataataatataattatttatacaataatatttaaataatatatttatttaatataattattatatttcacataaaagcaatagttccagtgttacaaattgtaggcaa

SEQ ID NO: 24 - DNA, 5460 bp, Artificial Sequence
  Synthetic
ctcgaggtctcaagataagaatgactgctgtaactcaaatccaccaaagctatttgtgttagaatgctttcctttggtaataacataataccacagagtgagtgaatgtatcaagcaaagtactcactcataatctctccacccaaatgactttgtcttctaaaattaaacccttcccagaggcctctccccttaataccatattgggctcttcacacttcttccaacatcgccttccatcctggcccttccaacctcccttctgtttgtgctaggaacagctcaaggcctcctatctaccacagagttacatggcttgccccttgccaaccccccagtaccacacagtgagtgcaaaatctcaccacattcagaacccagtcactattcaaatcatattttaacctttgcagtactgactacttttgattcatctaaacattactgaactttattctagaaaacatttaagaaatttgtagttaggttcatcctttgagaccttacatttaatttctttctatgtaaacggaaagcattgttcagtcccacgctcattatggcaacccacttccaagtacttcgtttactacgtgggctggaatcatacagttttctgttgtgcttgtgggagcagatccccctaacctctgctgatttttctcaccacttatcatacatttattacatgcatgcactgctgtgtgagtttctaaatacttgggtagcaattctctactattactttaattttcctacttgtctgcaaatacgaaaagtagcttgaaagaacttcagatctttgttgttatctgttgcaaacactccatttttctgttgtagcaaaaaaaaaaaaaaagacatccatagttgtcaatgagaatgcaagatacatacattctgcacctgtgtgctaacataagtggctgccctgtgactcagagattgcttgtccttctcctaagcctatccttttttgttactttggatacttttgttcaatgaatccagaaaaagtgtttttcagattcaccatgtgaccctcatttaaaacctgtaatccccctatggttaagttcctgcttttgtttctgttttctttctttcagtaaaaggaattgaacccagtccttccacttactatctgagcatatggctcttttagattatgatgttggtggtgttcattggtctcaccaaaatgctaaagaagccttcatcttctacttgtgggtagtctttacattcattactgcaagtttagtttatgtggtagtaccagatcctttgcttcttttgacttcatgcctacctaacagcgctctttcctttagttaagcttatgaaatagtgtttctctcatgtttcctctatattctctcttttgccttcctgtttcttcctgttgattccatcccattggagtgaaatcttatgatcttttggcatcaacaaagtgatctgcatccaaataattccacatctcattccatgttgactgtggatctatatatatatatatgtaatatgtatatatgtatatatgtatatatgtatatatgtatatatgtatatatgtatatatgtatatatgtatatatgtatatatgtatatatgtatatatgtatatatgtatatatgtatatatgtatatatgtatatatgtatatatgtatatatgtatatatgtatatatgtatatatgtatatatgtatatatgtatatatgtatatatgtatatatgtatatatgtatatatgtatatatgtatatatgtatatacgtatatatgcatatacgtatatatgtatatatgtatatatgtatatatgtatatatgtatatatgtatatatgtatatatgtatatatgtatgtatgtatgtatgtatgtatatatgtatatatgtatgtatgtatgtatgtatgtatgtatgtatatatgtatatatatatgtatgtatgtatgtatgtatgtatgtatatgtgtatatgtgtatatgtgtatatgtgtatatgtgtatatatgtatatatgtatatatgtatatatgtatatgtgtatatgtgtatatgtgtatatatgtatatatgtatatatgtatatatgtatatatataacatagtattaaattatatatacatatataagtgaaatgtcacaatcttctagaacttgctctgtatgtccacttaacatggtagagtgagctatgtcagcattttctatttcctgtgaatcattctgtgtgttgccaagaagaaatatgatatattctgaggttatgaaatgatattttggtcatcatgtttctcatcctattttcatattacctaaatacttttgcttttaaaattattattattaataataatataattatttatacaataatatttaaataatatatttatttaatataattattatatttcacataaaagcaatagttccagtgttacaaattgtaggcaatgggctgttctgattatctaagttgggcccaggatatgtgctgaatagttaaagcacatgcccagcatgtatgagggtaaaaggatgggtggatgtagtgacccatttgtaatttaagccttagcaggcagaggtgtgacccatagtgcaaagtacatagtcattataaggtcatctatatcacaatctctggattagattgattgaacctgctcagtgaccaatgtgttagcaatatacaggaggatgataacatcaacgtcagaagacacattgaagggcttacaaatagtgcccatttactttaatacagaaaaattcaatgtaccctctaggcaatttcaacttttagtctcttggtaggatagtctacatttagaatggctaattcataaattagaaagcttcttcaccccctacttttctggttatttctctatgaatgtggtaggcatgagttagtacacatgtttccatgtacatgtgtttctatgtgtctgcatgcatatggtagaatgtactcatattctatgtacagttagaacaatatttatattgtcaaagaaatcaaaaggagtattataagcttcagaaataaggataagtttgaaatattcattgttttattttttacagtattttttcctttgagaattctatgtaaagtactttgaacatatttgccttcaactcctccctcactttcaccctctcttcattcctccctttcctttccactcaaagttgagattcctttatttatttatttatccttcaaatatcactggtactatccacatgatctcaggattgaggtctgctctgacgtgtcatcctgctttcatgcaatggccttataggtggaacaacattatgaactaaccagtaccccggagctcttgactctagctgcatatatatcaaaagatggcctagtcggccatcactggaaagagaggctcattggacttgcaaactttatatgccccagtacaggggaacaccagggccaaaaagggggagtgggtgggcaggggagtgggggtgggtggatatgggggacttttggtatagcattggaaatgtaaatgagttaaatacctaataaaaaatggaaaaaaaaagtttctaatgtgtgtttctagaaacttcctctcttaaagcaacaacatgtccatgagcaatatagaattgaagatcaccatcaaatcctctttattcctcattgtttccatcatgtactaccagacctctttaaagtgtagtacagtgtgttaggaaatgagcagattatcctgggtatgtgctaaattagctactgagtcaaaatacattttttgctgaacattaagtgtttggtcatttctgggcaaaagaaagaaagaaagaaagaaaagaaagaaagaaaggaaggaaggaaggaaggaaggaaggaaggaaggaaagaaggaaggaaagaaaaaatggatgtaaattgttctgacagcatctgtctgagtcaggcagtggaatgaaggaggaatcctagagaatgcacaggaaagcagcccaaggagagtgtgggctgaaaggcatcatgttagaaacatgcactcgatgacagaaccttgagaaaaaggaactcaagcaaaagcacttatttaaaattgtaaaacgcactttattcatagccatgggggatgtcaatattccaagcataagaatgatcagtttccaatcactgtgaacccccaaaacacaaagtgaaaacccactactttatttgatgagatttggggttgctctattaatttataaaatcagagtaagacacgatataaatgaaacgattgtagttctaaagcagcggcacttccctgaacagtgtcattttgacaagtaactgctaacatcttcaggtcacagcgactgaagaaaaagtagggaaagaaggctggctgtgctgtttgacattttcttttcttatctggtgacatgaagagaagctctgggtccccctactcttgttcatatatctgttgcttttatgctgcatcctgaggtttgaagaaatgcatttggcactgagaaaagatgaggagagaatgccttggacatggtcctaacatgctttggtactgagaaaagagagcagaggagatgacatagaataggagagataatttggcctattttggccttcatctgagtgatagattttacttaacaaatagaaacaaagttttacttataaacagaaccaatgacctgtgtcatctctgatatattgagctttgaattcagtgaaattatgaactaaatatatcactccataattttctaagagggctatttgtatagtttcagtgatagtgtgacaaagtgtaatctaaatttctaaaaagtaaaataagtagataaaatagtaggtagaatagtataataatagaataagtataggtatggactagaataaatagacaaaatagtagataaaatgctaatgattttgttgacagggtaatcatgaatatttttattatttagctaaagaaccaatgttcatgtactcaagaagtgtattgaggaacttaggaaattagtctgaacaggtgagagggtgcgccagagaacctgacagcttctggaacaggcggaagcacagaggcactgaggcagcaccctgtgtgggccggggacagccggccaccttccggaccggaggacaggtgcccgcccggctggggaggcgacctaagccacagcagcagcggtcgccatcttggtccgggacccgccgaacttaggaaattagtctgaacaggtgagagggtgcgccagagaacctgacagcttctggaacaggcagaagcacagaggcgctgaggcagcaccctgtgtgggccggggacagccggccaccttccggaccggaggacaggtgcccacccggctggggaggcggcctaagccacagcagcagcggtcgccatcttggtcccggg

SEQ ID NO: 25 - DNA, 220 bp, Artificial Sequence
  Synthetic
taggcaacagagtgagatcatgtgtcatatatatatatatatatatatatatatatatatatatatacacacacacacacatatatatatacacatatatatacgtatatatatatatgtatatatatacatatatatacatatatatatatacgtatatatatacgtatatatatatcaatgtaaattatttgggaaatttggtatgaatagtcttccc

SEQ ID NO: 26 - DNA, 134 bp, Artificial Sequence
  Synthetic
aaatacaaaaattagccaggtgtggtggcatgtgcctgtagtcctacctactcgggaggctgaggcacaagaatcgcttgaatgtgggaggtggaggttgcagtgacctgagatcgtgccactgcactccagcc

SEQ ID NO: 27 - DNA, 246 bp, Artificial Sequence
  Synthetic
tgtgaacacagatcataaaatcatatatcaagcagacaaataagtagtagtcacttatatgcttatacttgtaacttaaagtaaaagaattacaaaagcatatgacaaagactaattttaagatatcctaatttaaattgttttctaaaagtgtgtataccattttacctatcatatgaataatttagaaacatgtttataaaattaatgtccaaatccattcaaaagttttgtaatgcagatcac

SEQ ID NO: 28 - DNA, 3361 bp, Artificial Sequence
  Synthetic
agcgccgaattcgatccctttataaaaccacaatataatggagtgctataatttcaaacagtgtttggtctgctggcagagtggtcattctaacagcagtcacagtagagtagaaataagactgcagtatatctaaggcaaaaagctgaggtttcaggagcttgaaggtaaagaggaagaaagaaatgggaatgggaattggaaagacaaatatcgttaagagaaaattgcttttaggagaggggaaagaatctatgtgtacttaagactatggaatcaatcccatttaagctgggaaactagtttcatatataactaataaattttatttacagaatatctatttacctgatctaggcttcaagccaaagggactgtgtgaaaaaccatcagttctgtcatattcctaaaaaaaaattaaaaagttaaaaataaataaataataaaacttcttttctttcaaaataatcaaggtgcttattcacatccattccaatttggggaaatacttattttcctatgattagcgaagagaaaagtaacttgcatttcaattcaagttgatacatgtcacttttaagaggtcaactaatatttgctagttgagctaaccatataggctttaaatactttcatagtagaaagaaaatgaaaatcattagtgaactgtataaaatagatcatactttttgaaagaatcagactgaagtttccgaaaaaaagaagtaagcttcaatgaaaaggtaagtgaatttagcatttactcagcatctactatggacttaacacctaacagtagataatctgaaggcaaacatatttgtatagggactgcagaatgatagatgataaatatcatctcttctatttgaatgaatattttttcaaatctttcacacacagtggtttgctatggaaagatttgtagtacattaaacaaatctgaagatggagttagaaagcttaggctatgttttgagcacaacatataatttctctgtgattgtttcttcatctttcaaatgaggttactgtgaagattaaatgagataactaaatgatgataaaataatgtaatcttagcagcaccttatttaatctgtgcaacaactctgtgaagtgagtagggctcagcttcagtcacttctctgccatttattaactaagatagtttggaaagttacccatctcttcagctgtaaaatgatgaggatcatacctattttatggggctgcttttaggtacaaatatacaggcaagcactttgttaatactaaagcattacaccaattagttttactcttttccattcacacatgaaattaatgtaatcagaattctgtagattacctaaatcttctgttaacacgtgatatgcagttcaggttaaatgtcagttgagttaccaaagcacatacatactcaccaccctatccaaatctacaagcctcccagtttgtcttcactattttggttaaattaatatgaattcctagatgaaaatttcactgatccaaatgaaataaaaaatatattacaaaactcacacctgtaatctcaacattttgggaggccaaggcaggtagatcacttgaggccaggagttcaagaccagcctgatcaacatggtgaaaccctgtctctactaaaatacaaaaattagccaggtgtggtggcatgtgcctgtagtcctacctactcgggaggctgaggcacaagaatcgcttgaatgtgggaggtggaggttgcagtgacctgagatcgtgccactgcactccagcctaggcaacagagtgagatcatgtgtcatatatatatatatatatatatatatatatatatatatatacacacacacacacatatatatatacacatatatatacgtatatatatatatgtatatatatacatatatatacatatatatatatacgtatatatatacgtatatatatatcaatgtaaattatttgggaaatttggtatgaatagtcttccctgtgaacacagatcataaaatcatatatcaagcagacaaataagtagtagtcacttatatgcttatacttgtaacttaaagtaaaagaattacaaaagcatatgacaaagactaattttaagatatcctaatttaaattgttttctaaaagtgtgtataccattttacctatcatatgaataatttagaaacatgtttataaaattaatgtccaaatccattcaaaagttttgtaatgcagatcacccacaacaacaaagaatcctagcctattaaaaaagcaacaccacctacatataatgaaatattagcagcatctatgtaaccaaagttacacagtgaatttgggccatccaacactttgagcaaagtgttgaattcatcaaatgaatgtgtaatcatttacttactaatgccaatacactttaaggtaatcttaagtagaagagatagagtttagaattttttaaatttatctcttgttgtaaagcaatagacttgaataaataaattagaagaatcagtcattcaagccaccagagtatttgatcgagatttcacaaactctaactttctgatacccattctcccaaaaacgtgtaacctcctgtcgataggaacaacccactgcagggatgtttctcgtggaaaaaggaaatttcttttgcattggtttcagacctaactggttacaagaaaaaccaaaggccattgcacaatgctgaagtacttttttcaaatttaaaatttgaaagttgttcttaaaatctatcatttattttaaaatacggatgaatgagaaagcatagatttgataaagtgaattcttttctgcaatctacagacacttccaaaaatcactacagacactacagacactacagaaaatcataaataaacaagtgctagtatcaatatttttaccaaaaaatggcattcttagaattttttataggctagaaggtttgtacaaactaatctgccacggattttaaaatatgagtgaataaattatattgcaaaaaaaatcaggttacagagaactggcaaggaagactcttatgtaaaacacagaaaacatacaaaacgtatttttaagacaaataaaaacagaacttgtacctcagatgatactggagattgtgttgacatattagcattatcactgtcttgctaaaacataaaaataaaaagatggaagatgaaattacaatacaaatgatgatttaaacatataaaaggaaaataaaaattgttctgaccaactactaaaggaagacctactaaagatatgccatccagcacattgccactctacatgtggtctgtaaaccagcagcataggcggccgcattagc

SEQ ID NO: 29 - DNA, 143 bp, Artificial Sequence
  Synthetic
attcaacagctgaatcctaaattgcaaactcagtggctaataacaactttgaacaatgagcaccttatacacgctactgtattttcttttctttcttttttttttttttttttttttttaaaccgggtagcagtgagagaggt

SEQ ID NO: 30 - DNA, 64 bp, Artificial Sequence
  Synthetic
tgtagtcattttgcaatccttaaagctgaattgtgcaatgagctcgatgaaggaagatactatc

SEQ ID NO: 31 - DNA, 73 bp, Artificial Sequence
  Synthetic
ttctttaagtgccttggggcgaggagtccggaataagaagacttctttgggttttaaagtgtaggataagcaa

SEQ ID NO: 32 - DNA, 1697 bp, Artificial Sequence
  Synthetic
agccctgcccccatccgacctccgccctcgttggcttcgcaacgctgtggtctctgtggccagtagagggcacacttactttactttcacaaatccgagagccacaacccgggtggtggggggtgagggggcggggaaagagtctctgcagcaaaacgcagactagggattggtggctcttggtgtttgaggcaaaatcctagaggctgtagtcattttgcaatccttaaagctgaattgtgcaatgagctcgatgaaggaagatactatcattcaacagctgaatcctaaattgcaaactcagtggctaataacaactttgaacaatgagcaccttatacacgctactgtattttcttttctttcttttttttttttttttttttttttaaaccgggtagcagtgagagaggtttctttaagtgccttggggcgaggagtccggaataagaagacttctttgggttttaaagtgtaggataagcaaatcccgagggaatatgcattatataataaatctagaaccaatgcacagagcaaaagactcatgtttctggttggttaataagctagattatcgtgtatatataaagtgtgtatgtatacgtttggggattgtacagaatgcacagcgtagtattcaggaaaaaggaaactgggaaattaatgtataaattaaaatcagcttttaattagcttaacacacacatacgaaggcaaaaatgtaacgttactttgatctgatcagggccgacttttttttttaagtgcataattacgattccagtaataaaaggggaaagcttgggtttgtcctgggaggaaggggttaacggttttctttattctagggtctctgcaggctccccagatctgggttggcaattcactcctccccctttctgggaagtccgggttttccccaaccccccaattcatggcatattctcgcgtctagcgccttgattttccccaccccagctcctaaaccagagtctgctgcaaactggctccacaggggcaaagaggatttgcctcttgtgaaaaccgactgtggccctggaactgtgtggaggtgtatggggtgtagaccggcagagactcctcccggaggagccgggtagagcgcacccgccgccactttactggactgcgcagggagacctacaggggaaagagccgcctccacaccacccgccgggtggaagtccgaaccggaggtgctggagtgtgtgtgtgggggggggggggaatctgccttttggcagcaaattgggggggggggtcgttctggaaagaatgtgcccagtcaacataactgtacgaccaaaggcaaaatacacaatgccttccccgcgagatggagtggctgtttatccctaagtggctctccaagtatacgtggcagtgagttgctgagcaattttaataaaattccagacatcgtttttcctgcatagacctcatctgcggttgatcaccctctatcactccacacactgagcgggggctcctagataactcattcgttcgtccttccccctttctaaattctgttttccccagccttagagagacgcctggccgcccgggacgtgcgtgacgcggtccagggtacatggcgtattgtgtggagcgaggcagctgttccacctgcggtgactgatatacgcagggcaagaacacagttcagccga

SEQ ID NO: 33 - DNA, 146 bp, Artificial Sequence
  Synthetic
tcacagacactacagaatgttttggagattatgtaatatttaaaatattcaaattatactaaaaatgtatgtaaaatgtattgaacataggcaagtttcaatacatagattttgagtgaatgcttgcaactttggttccattctct

SEQ ID NO: 34 - DNA, 77 bp, Artificial Sequence
  Synthetic
tctgactctgcactctgcaacctactctaatattacatatgataacatgagtctatgcagctgttctctatagatat

SEQ ID NO: 35 - DNA, 110 bp, Artificial Sequence
  Synthetic
ctacttccttaaggtggtgtccaagagtacatttttataaataaaaagttatagtacactcctaagggcagcaagtagaaaacgtgctagggagactcgatctcactttg

SEQ ID NO: 36 - DNA, 2195 bp, Artificial Sequence
  Synthetic
aagcttccttggaattaatggtcagataaggagctctagcaatatcactttaaatgcttaatatacaatatttagaaaaccttatgattgtaaagagcttaaaaaagatgtgaaagaacaatcactaaagcattgacaacatatgtgtgttagtgaacaatatgtaccaaaatggacagatgagaggtgtacattggggtgtgagttgataatccagcagactgtgggactagagggtctacgaaaaacaaaggaagaacatacaaacaaattttaaaacactgtctttcaacactaaaactgttggaatagagagcaagaatacatattggattcacattcagtttatttctcagattcagactagtgctctgactctgcactctgcaacctactctaatattacatatgataacatgagtctatgcagctgttctctatagatattcacagacactacagaatgttttggagattatgtaatatttaaaatattcaaattatactaaaaatgtatgtaaaatgtattgaacataggcaagtttcaatacatagattttgagtgaatgcttgcaactttggttccattctctctacttccttaaggtggtgtccaagagtacatttttataaataaaaagttatagtacactcctaagggcagcaagtagaaaacgtgctagggagactcgatctcactttggaatctatcctgggagacaaatgcctctacaaatggattagagaagacagttttaaagaggaagataatcaggtaaaatctggggttttatgagagaaagaaagaggtagaagaaaaaatttcaagctcgaacatcggatcaggtggcacaatgcggtcaatgcctgcaaactcagggtaagtattattctccctgtttacagttccgtggaggagaagtgacttgcctgtggtcatacaacagagcaaagaaaaggcttgagctagaactcaggcctttgttaggtctccccttcctcctagcacattggcaaattgcatgaggaaagtagaggtacagttgagttcatgtacaacaataaggcattcaggtaaagtgaatgagggcagaagttttatgatttagggaaggtgtaagacaggaaaatatctttgttcccaattaagaaagagatcccttgaccatcagttagagattcccccaagtccctctttgccataagtcactgaaactgagatccaaggcatggcttctgtgagtcaggagagcttaacccagaggagagatttcagaacaggatatttcctattttgagtatcctgctcatgccagtcatggataaatttgcatctggcttaagaaattactggatcagcattgttttgggtagtttcacttcctgctgggtggggtagcaggctctataaagagatcctctgctgcacgactcttaaacccctggtacctgagcactgatctgccttggagaacctggtgagtcggcttccttgagttcctctgttctttgtgccctgaaatgttgagtttaatctgaatatggcaagtttggtggatccaatcctatgaaaattgacttgatgctacttagtggatgaaaatttaagattagagcacaattatatgctattttagctttcttttgttatacaggtaggtatccatatggacagagaagttaaggggtaacctttgatatgaagaagaaaaaagaacaaagtatttttctttattctcttgctttctagtgtcctttacaaaggtttgtgtcttagcaggtgtgaaagactacaattctccctgagcagccctttgctctatgcccaagtcagcccacttggactttataacagataatgatgataggaatagcatattagattgcccagggtgtctgaacttgtgactgcctttcttgaattggttattttcagggaaataagatgcttgattctttataacagagataatttatttggaaaaattgtatgagaaaacacaggatttcctagggacaatgaagcaatttgttaaagtggaagggagaaaccagaaagtcttgaaaaggtaattaagaatttaaataatttcttggagattggagaaataatatgccatggtattacacaagctttggcttctctctctggaggattcccttcccacgaacactgttgtatcatttctttcaga